European Patent Specification EP 3 450 562 B1, published July 19, 2023. Title: RECOMBINANT CORYNEBACTERIUM GLUTAMICUM FOR THE PRODUCTION OF FUCOSYLLACTOSE AND METHOD FOR THE PRODUCTION OF 2'-FUCOSYLLACTOSE THEREFROM. Applicant: Seoul National University R&DB Foundation. The sequence listing filed with the application follows.

SEQUENCE LISTING (6 sequences)

SEQ ID NO: 1 - DNA, 1377 bp, Corynebacterium glutamicum ATCC 13032
atgcgtacccgtgaatctgtcacggctgtaattaaggcgtatgacgtccgtggtgttgttggtgtcgatattgatgctgatttcatttctgagactggcgctgcctttggtcggctcatgcgtagtgagggtgaaaccaccgttgctattggccatgacatgcgtgattcctcccctgaattggccaaggcgtttgccgatggcgtgactgcacagggtttggatgttgttcatttgggactgacttctactgatgagctgtactttgcgtccggaaccttgaagtgtgctggtgcgatgtttactgcgtcgcataaccccgctgagtacaacggcatcaagttgtgtcgtgcgggtgctcgtccggtcggtcaggattctggtttggccaacatcattgatgatctggttgagggtgttccagcgtttgatggtgagtcaggttcggtttctgagcaggatttgctgagcgcatatgccgagtacctcaatgagcttgttgatctgaagaacatccgcccgttgaaggttgctgtggatgcggcaaacggcatgggtgggttcactgtccctgaggtattcaagggtctgccacttgatgttgcgccactgtattttgagcttgacggcaatttccccaaccatgaggccaatcctctggagcctgccaacctggttgatttgcagaagtttaccgtagagaccggatctgatatcggtttggcgttcgacggcgatgcggatcgttgcttcgtggtcgatgagaagggccagccagtcagcccttcggcgatctgtgcgatcgtagcggagcgttacttggagaagcttccgggttccaccatcatccacaacctgattacctctaaggctgtgcctgaggtgattgctgaaaacggtggcactgcggtgcgtactcgcgtgggtcactccttcatcaaggcgaagatggcagagaccggtgcggcctttggtggcgagcactctgcgcactactacttcactgagttcttcaatgcggactccggcattttggctgcgatgcacgtgctggctgcgctgggaagccaggaccagccactcagtgagatgatggctaggtataaccggtacgttgcttcaggcgagttgaactcccgtttggctaatgcagaggcgcagcaagagcgcacccaggctgtgctcgatgcgttcgctgatcgcaccgagtccgtggacacccttgacggcgtgactgtggaactcaaggacacctccgcgtggttcaacgtgcgtgcgtccaacaccgagccgctgcttcgcctcaatgttgaagctgcatcgaaggaagaagtcgatgcgttggtagcggagattctagggattatccgcgcataa

SEQ ID NO: 2 - DNA, 1089 bp, Corynebacterium glutamicum ATCC 13032
atgactttaactgacaacagcaaaaacgttgatgctgtcatcttggtcggtggcaaaggtacccgactgcgccccctgaccgtcaatactccaaagccaatgctgccaactgctggccacccattcttgacccaccttttggcccgcatcaaggccgcaggcatcacacacgtcgtgctgggaacgtcattcaaagctgaagtcttcgaggaatacttcggagatggctccgaaatgggcttggaaattgaatatgtcgtcgaggatcagcctttgggcactggtggtggcatccgaaacgtctacgacaagctgcgtcacgatactgcgattgtgttcaacggcgatgtgctctccggtgcggatctcaacagcattctggacacccaccgcgaaaaggacgcagatctgaccatgcatctcgtgcgcgtagctaaccctcgtgcgtttggttgcgtccccaccgatgaggatggtcgcgtcagcgaattccttgaaaagaccgaagatccaccaaccgatcagatcaacgccggctgctacgtgttcaagaaggaactcatcgagcagatcccggcaggccgagcagtttccgtcgagcgcgaaaccttccctcagctgttggaagaaggcaagcgagtcttcggccacgtcgacgcttcctactggcgcgacatgggcaccccaagcgacttcgtccgcggctcggctgacctggtccgcggcattgcgtactccccattgctcgaaggcaaaacaggagagtcgcttgtcgacgcctccgccggcgttcgcgacggcgtcctgctgctcggcggaaccgtagtcggccgcggcactgagatcggtgccggctgccgcgttgacaacactgttattttcgacggcgtcaccattgaaccaggtgcggtcattgaaaattccatcatttcctcgggagcacgcatcggtgctaatgcgcacatctccggttgcatcattggcgagggcgcacaggttggtgctcggtgtgaactcaacgcagggatgcgcgtcttcccaggcgttgtgatcccagacagcggaattcgtttttcgtctgatcagtag

SEQ ID NO: 3 - DNA, 2090 bp, E.coli K-12 MG1655
atgtcaaaagtcgctctcatcaccggtgtaaccggacaagacggttcttacctggcagagtttctgctggaaaaaggttacgaggtgcatggtattaagcgtcgcgcatcgtcattcaacaccgagcgcgtggatcacatttatcaggatccgcacacctgcaacccgaaattccatctgcattatggcgacctgagtgatacctctaacctgacgcgcattttgcgtgaagtacagccggatgaagtgtacaacctgggcgcaatgagccacgttgcggtctcttttgagtcaccagaatataccgctgacgtcgacgcgatgggtacgctgcgcctgctggaggcgatccgcttcctcggtctggaaaagaaaactcgtttctatcaggcttccacctctgaactgtatggtctggtgcaggaaattccgcagaaagagaccacgccgttctacccgcgatctccgtatgcggtcgccaaactgtacgcctactggatcaccgttaactaccgtgaatcctacggcatgtacgcctgtaacggaattctcttcaaccatgaatccccgcgccgcggcgaaaccttcgttacccgcaaaatcacccgcgcaatcgccaacatcgcccaggggctggagtcgtgcctgtacctcggcaatatggattccctgcgtgactggggccacgccaaagactacgtaaaaatgcagtggatgatgctgcagcaggaacagccggaagatttcgttatcgcgaccggcgttcagtactccgtgcgtcagttcgtggaaatggcggcagcacagctgggcatcaaactgcgctttgaaggcacgggcgttgaagagaagggcattgtggtttccgtcaccgggcatgacgcgccgggcgttaaaccgggtgatgtgattatcgctgttgacccgcgttacttccgtccggctgaagttgaaacgctgctcggcgacccgaccaaagcgcacgaaaaactgggctggaaaccggaaatcaccctcagagagatggtgtctgaaatggtggctaatgacctcgaagcggcgaaaaaacactctctgctgaaatctcacggctacgacgtggcgatcgcgctggagtcataagcatgagtaaacaacgagtttttattgctggtcatcgcgggatggtcggttccgccatcaggcggcagctcgaacagcgcggtgatgtggaactggtattacgcacccgcgacgagctgaacctgctggacagccgcgccgtgcatgatttctttgccagcgaacgtattgaccaggtctatctggcggcggcgaaagtgggcggcattgttgccaacaacacctatccggcggatttcatctaccagaacatgatgattgagagcaacatcattcacgccgcgcatcagaacgacgtgaacaaactgctgtttctcggatcgtcctgcatctacccgaaactggcaaaacagccgatggcagaaagcgagttgttgcagggcacgctggagccgactaacgagccttatgctattgccaaaatcgccgggatcaaactgtgcgaatcatacaaccgccagtacggacgcgattaccgctcagtcatgccgaccaacctgtacgggccacacgacaacttccacccgagtaattcgcatgtgatcccagcattgctgcgtcgcttccacgaggcgacggcacagaatgcgccggacgtggtggtatggggcagcggtacaccgatgcgcgaatttctgcacgtcgatgatatggcggcggcgagcattcatgtcatggagctggcgcatgaagtctggctggagaacacccagccgatgttgtcgcacattaacgtcggcacgggcgttgactgcactatccgcgagctggcgcaaaccatcgccaaagtggtgggttacaaaggccgggtggtttttgatgccagcaaaccggatggcacgccgcgcaaactgctggatgtgacgcgcctgcatcagcttggctggtatcacgaaatctcactggaagcggggcttgccagcacttaccagtggttccttgagaatcaagaccgctttcgggggtaa

SEQ ID NO: 4 - DNA, 916 bp, Helicobacter pylori ATCC 700392
aaggagatatacaatggcttttaaggtggtgcaaatttgcggagggcttgggaatcaaatgtttcaatacgctttcgctaaaagtttgcaaaaacactctaatacgcctgtgctgttagatatcacttcttttgattggagcgataggaaaatgcaattagaacttttccctattgatttgccctatgcgagcgcgaaagaaatcgctatagctaaaatgcaacacctccccaagctagtaagagacgcgctcaaatgcatgggatttgatagggtgagtcaagaaatcgtttttgaatacgagcctaaattgctaaagccaagccgcttgacttatttttttggctatttccaagatccacgatactttgatgctatatcccctttaatcaagcaaaccttcactctaccccccccccccgaaaataataagaataataataaaaaagaggaagaatatcagtgcaagctttctttgattttagccgctaaaaacagcgtgtttgtgcatataagaagaggggattatgtggggattggctgtcagcttggtattgactatcaaaaaaaggcgcttgagtatatggcaaagcgcgtgccaaacatggagctttttgtgttttgcgaagacttagaattcacgcaaaatcttgatcttggctacccttttatggacatgaccactagggataaagaagaagaggcgtattgggacatgctgctcatgcaatcttgtcagcatgccattatcgctaatagcacttatagctggtgggcggcctatttgatagaaaatccagaaaaaatcattattggccccaaacactggctttttgggcatgagaatatcctttgtaaggagtgggtgaaaatagaatcccattttgaggtaaaatcccaaaagtataacgcttaa

SEQ ID NO: 5 - DNA, 3335 bp, E.coli BL21star(DE3)
accatcgaatggcgcaaaacctttcgcggtatggcatgatagcgcccggaagagagtcaattcagggtggtgaatgtgaaaccagtaacgttatacgatgtcgcagagtatgccggtgtctcttatcagaccgtttcccgcgtggtgaaccaggccagccacgtttctgcgaaaacgcgggaaaaagtggaagcggcgatggcggagctgaattacattcccaaccgcgtggcacaacaactggcgggcaaacagtcgttgctgattggcgttgccacctccagtctggccctgcacgcgccgtcgcaaattgtcgcggcgattaaatctcgcgccgatcaactgggtgccagcgtggtggtgtcgatggtagaacgaagcggcgtcgaagcctgtaaagcggcggtgcacaatcttctcgcgcaacgcgtcagtgggctgatcattaactatccgctggatgaccaggatgccattgctgtggaagctgcctgcactaatgttccggcgttatttcttgatgtctctgaccagacacccatcaacagtattattttctcccatgaagacggtacgcgactgggcgtggagcatctggtcgcattgggtcaccagcaaatcgcgctgttagcgggcccattaagttctgtctcggcgcgtctgcgtctggctggctggcataaatatctcactcgcaatcaaattcagccgatagcggaacgggaaggcgactggagtgccatgtccggttttcaacaaaccatgcaaatgctgaatgagggcatcgttcccactgcgatgctggttgccaacgatcagatggcgctgggcgcaatgcgcgccattaccgagtccgggctgcgcgttggtgcggatatctcggtagtgggatacgacgataccgaagacagctcatgttatatcccgccgttaaccaccatcaaacaggattttcgcctgctggggcaaaccagcgtggaccgcttgctgcaactctctcagggccaggcggtgaagggcaatcagctgttgcccgtctcactggtgaaaagaaaaaccaccctggcgcccaatacgcaaaccgcctctccccgcgcgttggccgattcattaatgcagctggcacgacaggtttcccgactggaaagcgggcagtgagcgcaacgcaattaatgtgagttagctcactcattaggcaccccaggctttacactttatgcttccggctcgtatgttgtgtggaattgtgagcggataacaatttcacacaggaaacagctatgtactatttaaaaaacacaaacttttggatgttcggtttattctttttcttttacttttttatcatgggagcctacttcccgtttttcccgatttggctacatgacatcaaccatatcagcaaaagtgatacgggtattatttttgccgctatttctctgttctcgctattattccaaccgctgtttggtctgctttctgacaaactcgggctgcgcaaatacctgctgtggattattaccggcatgttagtgatgtttgcgccgttctttatttttatcttcgggccactgttacaatacaacattttagtaggatcgattgttggtggtatttatctaggcttttgttttaacgccggtgcgccagcagtagaggcatttattgagaaagtcagccgtcgcagtaatttcgaatttggtcgcgcgcggatgtttggctgtgttggctgggcgctgtgtgcctcgattgtcggcatcatgttcaccatcaataatcagtttgttttctggctgggctctggctgtgcactcatcctcgccgttttactctttttcgccaaaacggatgcgccctcttctgccacggttgccaatgcggtaggtgccaaccattcggcatttagccttaagctggcactggaactgttcagacagccaaaactgtggtttttgtcactgtatgttattggcgtttcctgcacctacgatgtttttgaccaacagtttgctaatttctttacttcgttctttgctaccggtgaacagggtacgcgggtatttggctacgtaacgacaatgggcgaattacttaacgcctcgattatgttctttgcgccactgatcattaatcgcatcggtgggaaaaacgccctgctgctggctggcactattatgtctgtacgtattattggctcatcgttcgccacctcagcgctggaagtggttattctgaaaacgctgcatatgtttgaagtaccgttcctgctggtgggctgctttaaatatattaccagccagtttgaagtgcgtttttcagcgacgatttatctggtctgtttctgcttctttaagcaactggcgatgatttttatgtctgtactggcgggcaatatgtatgaaagcatcggtttccagggcgcttatctggtgctgggtctggtggcgctgggcttcaccttaatttccgtgttcacgcttagcggccccggcccgctttccctgctgcgtcgtcaggtgaatgaagtcgcttaagcaatcaatgtcggatgcggcgcgagcgccttatccgaccaacatatcataacggagtgatcgcattgaacatgccaatgaccgaaagaataagagcaggcaagctatttaccgatatgtgcgaaggcttaccggaaaaaagacttcgtgggaaaacgttaatgtatgagtttaatcactcgcatccatcagaagttgaaaaaagagaaagcctgattaaagaaatgtttgccacggtaggggaaaacgcctgggtagaaccgcctgtctatttctcttacggttccaacatccatataggccgcaatttttatgcaaatttcaatttaaccattgtcgatgactacacggtaacaatcggtgataacgtactgattgcacccaacgttactctttccgttacgggacaccctgtacaccatgaattgagaaaaaacggcgagatgtactcttttccgataacgattggcaataacgtctggatcggaagtcatgtggttattaatccaggcgtcaccatcggggataattctgttattggcgcgggtagtatcgtcacaaaagacattccaccaaacgtcgtggcggctggcgttccttgtcgggttattcgcgaaataaacgaccgggataagcactattatttcaaagattataaagttgaatcgtcagtttaaattataaaaattgcctgatacgctgcgcttatcaggcctacaagttcagcgatctacattagccgcatccggcatgaacaaagcgcaggaacaagcgtcgcatcatgcctctttgacccacagc

SEQ ID NO: 6 - DNA, 903 bp, Artificial Sequence
  COfucT2
atggcgtttaaagtggtgcaaatttgcggaggcttgggtaaccaaatgtttcagtacgccttcgctaaaagtttgcaaaagcattccaacacgccggtgctgctcgatatcactagctttgattggtctgatcgcaaaatgcaactggaactttttccgattgacttgccatacgcctcggcgaaagagatcgcgatcgctaaaatgcagcacctcccgaagctagtccgcgatgcactgaagtgcatgggcttcgaccgcgtgtctcaagaaatcgttttcgaatacgagccgaagcttctcaagccaagccgcctcacttatttcttcggctacttccaggacccacgatactttgatgctatctcccctttaatcaagcaaaccttcaccctgccacccccccccgaaaacaacaagaataataataagaaagaggaagagtatcagtgcaagctttcactcatcctcgccgctaagaatagcgtgtttgttcacatccgtcgcggtgactatgtcggcattggctgtcagctgggtattgattaccagaagaaggctcttgagtacatggcaaagcgcgtgccaaacatggaacttttcgtgttttgcgaagatctggaattcacacagaaccttgaccttggataccctttcatggatatgaccacccgtgacaaggaggaagaagcgtactgggacatgctgctcatgcagtcttgccagcacgccattatcgcaaactccacctattcgtggtgggcagcgtacttgatcgagaacccagaaaagattattattggccctaaacactggttgttcgggcacgaaaacatcctgtgtaaagagtgggtgaaaatcgaatcccatttcgaggtcaaatcccagaagtataacgcataa